European Patent Application EP 4 520 397 A1, published March 12, 2025. Title: Polypeptides comprising histone code reader domains and uses thereof. Applicant: KOREA ADVANCED INSTITUTE OF SCIENCE AND TECHNOLOGY. The sequence listing filed with the application follows.

SEQUENCE LISTING (6 sequences)

SEQ ID NO: 1 - protein, 364 aa, synthetic construct
  REGION 1..364: note = Synthetic Sequence
MSSSIEQKKGSTRQRKCGFCKSNRDKECGQLLISENQKVAAHHKCMLFSSALVSSHSDNESLGGFSIEDVQKEIKRGTKLMCSLCHCPGATIGCDVKTCHRTYHYHCALHDKAQIREKPSQGIYMVYCRKHKKTAHNSEADLEESFNEHELEPSSPKTKKKSRKGRPRKTNLKGLPEDSRSTSSHGTDEMESSSYRDRSPHRSSPNDTRPKCGFCHVGEEENEARGKLHIFNAKKAAAHYKCMLFSSGTVQLTTTSRAEFGDFDIKTVLQEIKRGKRMKCTLCSQPGATIGCEIKACVKTYHYHCGVQDKAKYIENMSRGIYKLYCKNHSGNDERDEEDEERESKSRGRVAIDQQLTQQQLNGN

SEQ ID NO: 2 - protein, 115 aa, synthetic construct
  REGION 1..115: note = Synthetic Sequence
CGFCKSNRDKECGQLLISENQKVAAHHKCMLFSSALVSSHSDNESLGGFSIEDVQKEIKRGTKLMCSLCHCPGATIGCDVKTCHRTYHYHCALHDKAQIREKPSQGIYMVYCRKH

SEQ ID NO: 3 - protein, 122 aa, synthetic construct
  REGION 1..122: note = Synthetic Sequence
TRPKCGFCHVGEEENEARGKLHIFNAKKAAAHYKCMLFSSGTVQLTTTSRAEFGDFDIKTVLQEIKRGKRMKCTLCSQPGATIGCEIKACVKTYHYHCGVQDKAKYIENMSRGIYKLYCKNH

SEQ ID NO: 4 - protein, 56 aa, synthetic construct
  REGION 1..56: note = Synthetic Sequence
YCDFCLGGSNMNKKSGRPEELVSCADCGRSGHPTCLQFTLNMTEAVKTYKWQCIEC

SEQ ID NO: 5 - protein, 61 aa, synthetic construct
  REGION 1..61: note = Synthetic Sequence
SCILCGTSENDDQLLFCDDCDRGYHMYCLNPPVAEPPEGSWSCHLCWELLKEKASAFGCQA

SEQ ID NO: 6 - protein, 531 aa, synthetic construct
  REGION 1..531: note = Synthetic Sequence
MSSSIEQKKGSTRQRKCGFCKSNRDKECGQLLISENQKVAAHHKCMLFSSALVSSHSDNESLGGFSIEDVQKEIKRGTKLMCSLCHCPGATIGCDVKTCHRTYHYHCALHDKAQIREKPSQGIYMVYCRKHKKTAHNSEADLEESFNEHELEPSSPKTKKKSRKGRPRKTNLKGLPEDSRSTSSHGTDEMESSSYRDRSPHRSSPNDTRPKCGFCHVGEEENEARGKLHIFNAKKAAAHYKCMLFSSGTVQLTTTSRAEFGDFDIKTVLQEIKRGKRMKCTLCSQPGATIGCEIKACVKTYHYHCGVQDKAKYIENMSRGIYKLYCKNHSGNDERDEEDEERESKSRGRVAIDQQLTQQQLNGNHMGSGGGGPGTRPKCGFCHVGEEENEARGKLHIFNAKKAAAHYKCMLFSSGTVQLTTTSRAEFGDFDIKTVLQEIKRGKRMKCTLCSQPGATIGCEIKACVKTYHYHCGVQDKAKYIENMSRGIYKLYCKNHSGNDERDEEDEERESKSRGRVAIDQQLTQQQLNGN